European Patent Specification EP 3 457 868 B1, published April 15, 2026. Title: Flavour generation in food. Applicant: NESTEC S.A. The sequence listing filed with the application follows.

SEQUENCE LISTING (1 sequence)

SEQ ID NO: 1 - protein, 533 aa, Kluyveromyces lactis
MLARVFPKRSSFAANHTIKTTVTVKTRRSSRFYSKLSIDNNNLRKIKMSSSVAEKNFESLFQKIDELKPRFIERLAKAIEIPAVSGDETLRPQVIKKAHYLAGELKKLGFSDIQMKELGTQPPPVADPNLQLPPVILARYGNDPDKKTVLVYGHYDVQPASLEDGWNTDPFKLVVNEEKQIMYGRGVSDDSGPVKGWLNVVEAHRELGLDLPVNLITCLEGMEESGSIGLDKLIAEEAEGYFRTVDTVCISDNYWLGTQKPVLTYGLRGCNYYQIIIEGPGADLHSGIFGGSISEPMIDLVQVMSTLVDTKGNILIDGIKEMVAPVLETEDALYDKIDYSVDEFNAASGSKTALYDNKKDILMHRWRYPSLSIHGVEGAFHGSGAKTVIPSKVIGKFSIRTVPNIESAKLDQFVIDHCNKAFAKLQSPNKFKAELIHDGNYWVSDPFNASFSAAAKATKVVWGVEPDFTREGGSIPITLTFEQELKSNVLLLPMGRGDDGAHSINEKLDLSNYFGGMKTMAAYLHYYAASEEK